European Patent Application EP 4 375 367 A1, published May 29, 2024. Title: Recombinant Protein of Nerve Growth Factor Mutant and Use Thereof. Applicant: SHANGHAI JIAO TONG UNIVERSITY SCHOOL OF MEDICINE. Application EP 22860539.0, filed August 24, 2022. The sequence listing filed with the application follows.

SEQUENCE LISTING (70 sequences)

SEQ ID NO: 1 - DNA, 723 bp, synthetic construct
  misc_feature 1..723: note = NGFwt optimized coding region sequence
  source 1..723: mol_type = other DNA
atgtccatgttgttctacactctgatcacagcttttctgatcggcatacaggcggaaccacactcagagagcaatgtccctgcaggacacaccatcccccaagcccactggactaaacttcagcattcccttgacactgcccttcgcagagcccgcagcgccccggcagcggcgatagctgcacgcgtggcggggcagacccgcaacattactgtggaccccaggctgtttaaaaagcggcgactccgttcaccccgtgtgctgtttagcacccagcctccccgtgaagctgcagacactcaggatctggacttcgaggtcggtggtgctgcccccttcaacaggactcacaggagcaagcggtcatcatcccatcccatcttccacaggggcgaattctcggtgtgtgacagtgtcagcgtgtgggttggggataagaccaccgccacagacatcaagggcaaggaggtgatggtgttgggagaggtgaacattaacaacagtgtattcaaacagtacttttttgagaccaagtgccgggacccaaatcccgttgacagcgggtgccggggcattgactcaaagcactggaactcatattgtaccacgactcacacctttgtcaaggcgctgaccatggatggcaagcaggctgcctggcggtttatccggatagatacggcctgtgtgtgtgtgctcagcaggaaggctgtgagaagagcc

SEQ ID NO: 2 - DNA, 723 bp, synthetic construct
  misc_feature 1..723: note = NGFmut optimized coding region sequence
  source 1..723: mol_type = other DNA
atgtccatgttgttctacacactgatcaccgccttcctgatcggcatccaggccgagcctcacagcgagtccaatgtgcccgccggccacaccatcccccaggctcattggaccaagctgcagcactccctggatacagccctgagaagagccagatccgcccctgccgccgccatcgctgctagagtggccggacagacaaggaacatcacagtggaccctagactgtttaagaagagaagactgaggagccccagagtgctgttctccacacagccccccagagaggccgccgacacacaggacctggatttcgaggtgggcggcgccgccccttttaacagaacacacagatccaagaggtccagctcccaccctatcttccacagaggcgagttcagcgtgtgcgactccgtgagcgtgtgggtgggcgacaagaccaccgccaccgacatcaagggcaaggaggtcatggtgctgggcgaggtgaacatcaataacagcgtgtttaagcagtactttttcgagaccaagtgcagagaccctaaccctgtggactccggctgtagaggcatcgactccaagcactggaatagctactgcaccacaacccacacattcgtgaaggccctgacaatggacggcaagcaggccgcctggtggttcatcagaatcgacaccgcctgtgtgtgtgtgctgagcagaaaggctgtgagaagagcc

SEQ ID NO: 3 - DNA, 762 bp, synthetic construct
  misc_feature 1..762: note = IGK19-NGFmut optimized sequence of coding region
  source 1..762: mol_type = other DNA
atggagacagacacactcctgctatgggtactgctgctctgggttccaggttccaccggagacgagcctcacagcgagtccaatgtgcccgccggccacaccatcccccaggctcattggaccaagctgcagcactccctggatacagccctgagaagagccagatccgcccctgccgccgccatcgctgctagagtggccggacagacaaggaacatcacagtggaccctagactgtttaagaagagaagactgaggagccccagagtgctgttctccacacagccccccagagaggccgccgacacacaggacctggatttcgaggtgggcggcgccgccccttttaacagaacacacagatccaagaggtccagctcccaccctatcttccacagaggcgagttcagcgtgtgcgactccgtgagcgtgtgggtgggcgacaagaccaccgccaccgacatcaagggcaaggaggtcatggtgctgggcgaggtgaacatcaataacagcgtgtttaagcagtactttttcgagaccaagtgcagagaccctaaccctgtggactccggctgtagaggcatcgactccaagcactggaatagctactgcaccacaacccacacattcgtgaaggccctgacaatggacggcaagcaggccgcctggagattcatcagaatcgacaccgcctgtgtgtgtgtgctgagcagaaaggccgtgagaagggcctacccgtacgacgtgccggactacgcctga

SEQ ID NO: 4 - DNA, 423 bp, synthetic construct
  misc_feature 1..423: note = IGK122-NGFmut optimized sequence of coding region
  source 1..423: mol_type = other DNA
atggagacagacacactcctgctatgggtactgctgctctgggttccaggttccaccggagactccagctcccaccctatcttccacagaggcgagttcagcgtgtgcgactccgtgagcgtgtgggtgggcgacaagaccaccgccaccgacatcaagggcaaggaggtcatggtgctgggcgaggtgaacatcaataacagcgtgtttaagcagtactttttcgagaccaagtgcagagaccctaaccctgtggactccggctgtagaggcatcgactccaagcactggaatagctactgcaccacaacccacacattcgtgaaggccctgacaatggacggcaagcaggccgcctggtggttcatcagaatcgacaccgcctgtgtgtgtgtgctgagcagaaaggctgtgagaagagcc

SEQ ID NO: 5 - DNA, 939 bp, synthetic construct
  misc_feature 1..939: note = IGK19-NGF-PDGFRmut optimized sequence of coding region
  source 1..939: mol_type = other DNA
atggagacagacacactcctgctatgggtactgctgctctgggttccaggttccaccggagacgagcctcacagcgagtccaatgtgcccgccggccacaccatcccccaggctcattggaccaagctgcagcactccctggatacagccctgagaagagccagatccgcccctgccgccgccatcgctgctagagtggccggacagacaaggaacatcacagtggaccctagactgtttaagaagagaagactgaggagccccagagtgctgttctccacacagccccccagagaggccgccgacacacaggacctggatttcgaggtgggcggcgccgccccttttaacagaacacacagatccaagaggtccagctcccaccctatcttccacagaggcgagttcagcgtgtgcgactccgtgagcgtgtgggtgggcgacaagaccaccgccaccgacatcaagggcaaggaggtcatggtgctgggcgaggtgaacatcaataacagcgtgtttaagcagtactttttcgagaccaagtgcagagaccctaaccctgtggactccggctgtagaggcatcgactccaagcactggaatagctactgcaccacaacccacacattcgtgaaggccctgacaatggacggcaagcaggccgcctggagattcatcagaatcgacaccgcctgtgtgtgtgtgctgagcagaaaggccgtgagaagggcctacccgtacgacgtgccggactacgcctgatacccgtacgacgtgccggactacgccaatgctgtgggccaggacacgcaggaggtcatcgtggtgccacactccttgccctttaaggtggtggtgatctcagccatcctggccctggtggtgctcaccatcatctcccttatcatcctcatcatgctttggcagaagaagccacgt

SEQ ID NO: 6 - DNA, 600 bp, synthetic construct
  misc_feature 1..600: note = IGK122-NGF-PDGFRmut optimized sequence of coding region
  source 1..600: mol_type = other DNA
atggagacagacacactcctgctatgggtactgctgctctgggttccaggttccaccggagactccagctcccaccctatcttccacagaggcgagttcagcgtgtgcgactccgtgagcgtgtgggtgggcgacaagaccaccgccaccgacatcaagggcaaggaggtcatggtgctgggcgaggtgaacatcaataacagcgtgtttaagcagtactttttcgagaccaagtgcagagaccctaaccctgtggactccggctgtagaggcatcgactccaagcactggaatagctactgcaccacaacccacacattcgtgaaggccctgacaatggacggcaagcaggccgcctggtggttcatcagaatcgacaccgcctgtgtgtgtgtgctgagcagaaaggctgtgagaagagcctacccgtacgacgtgccggactacgccaatgctgtgggccaggacacgcaggaggtcatcgtggtgccacactccttgccctttaaggtggtggtgatctcagccatcctggccctggtggtgctcaccatcatctcccttatcatcctcatcatgctttggcagaagaagccacgt

SEQ ID NO: 7 - DNA, 723 bp, synthetic construct
  misc_feature 1..723: note = BDNF19-NGFmut optimized coding region sequence
  source 1..723: mol_type = other DNA
atgaccatcctgttcctgacaatggtcattagctacttcggctgcatgaaggccgagcctcacagcgagtccaatgtgcccgccggccacaccatcccccaggctcattggaccaagctgcagcactccctggatacagccctgagaagagccagatccgcccctgccgccgccatcgctgctagagtggccggacagacaaggaacatcacagtggaccctagactgtttaagaagagaagactgaggagccccagagtgctgttctccacacagccccccagagaggccgccgacacacaggacctggatttcgaggtgggcggcgccgccccttttaacagaacacacagatccaagaggtccagctcccaccctatcttccacagaggcgagttcagcgtgtgcgactccgtgagcgtgtgggtgggcgacaagaccaccgccaccgacatcaagggcaaggaggtcatggtgctgggcgaggtgaacatcaataacagcgtgtttaagcagtactttttcgagaccaagtgcagagaccctaaccctgtggactccggctgtagaggcatcgactccaagcactggaatagctactgcaccacaacccacacattcgtgaaggccctgacaatggacggcaagcaggccgcctggtggttcatcagaatcgacaccgcctgtgtgtgtgtgctgagcagaaaggctgtgagaagagcc

SEQ ID NO: 8 - DNA, 744 bp, synthetic construct
  misc_feature 1..744: note = BDNF122-NGFmut optimized coding region sequence
  source 1..744: mol_type = other DNA
atgaccatcctgttcctgacaatggtcattagctacttcggctgcatgaaggccgcccccatgaaggaggccaacatcagaggccagggcggcctggcctaccccggagtgagaacacacggcacactggagtccgtgaacggccccaaggccggctccaggggactgacaagcctggccgataccttcgagcacgtgatcgaggagctgctggacgaggaccagaaggtgaggcccaatgaggagaataataaggacgccgacctgtacacctccagggtcatgctgagcagccaggtgcccctggagcccccactgctgttcctgctggaggagtacaagaattacctggacgccgccaatatgtccatgagagtgagaaggtccagctcccaccctatcttccacagaggcgagttcagcgtgtgcgactccgtgagcgtgtgggtgggcgacaagaccaccgccaccgacatcaagggcaaggaggtcatggtgctgggcgaggtgaacatcaataacagcgtgtttaagcagtactttttcgagaccaagtgcagagaccctaaccctgtggactccggctgtagaggcatcgactccaagcactggaatagctactgcaccacaacccacacattcgtgaaggccctgacaatggacggcaagcaggccgcctggtggttcatcagaatcgacaccgcctgtgtgtgtgtgctgagcagaaaggctgtgagaagagcc

SEQ ID NO: 9 - DNA, 726 bp, synthetic construct
  misc_feature 1..726: note = NGFwt coding region sequence
  source 1..726: mol_type = other DNA
atgtccatgttgttctacactctgatcacagcttttctgatcggcatacaggcggaaccacactcagagagcaatgtccctgcaggacacaccatcccccaagcccactggactaaacttcagcattcccttgacactgcccttcgcagagcccgcagcgccccggcagcggcgatagctgcacgcgtggcggggcagacccgcaacattactgtggaccccaggctgtttaaaaagcggcgactccgttcaccccgtgtgctgtttagcacccagcctccccgtgaagctgcagacactcaggatctggacttcgaggtcggtggtgctgcccccttcaacaggactcacaggagcaagcggtcatcatcccatcccatcttccacaggggcgaattctcggtgtgtgacagtgtcagcgtgtgggttggggataagaccaccgccacagacatcaagggcaaggaggtgatggtgttgggagaggtgaacattaacaacagtgtattcaaacagtacttttttgagaccaagtgccgggacccaaatcccgttgacagcgggtgccggggcattgactcaaagcactggaactcatattgtaccacgactcacacctttgtcaaggcgctgaccatggatggcaagcaggctgcctggcggtttatccggatagatacggcctgtgtgtgtgtgctcagcaggaaggctgtgagaagagcctga

SEQ ID NO: 10 - DNA, 726 bp, synthetic construct
  misc_feature 1..726: note = NGFmut coding region sequence
  source 1..726: mol_type = other DNA
atgtccatgttgttctacactctgatcacagcttttctgatcggcatacaggcggaaccacactcagagagcaatgtccctgcaggacacaccatcccccaagcccactggactaaacttcagcattcccttgacactgcccttcgcagagcccgcagcgccccggcagcggcgatagctgcacgcgtggcggggcagacccgcaacattactgtggaccccaggctgtttaaaaagcggcgactccgttcaccccgtgtgctgtttagcacccagcctccccgtgaagctgcagacactcaggatctggacttcgaggtcggtggtgctgcccccttcaacaggactcacaggagcaagcggtcatcatcccatcccatcttccacaggggcgaattctcggtgtgtgacagtgtcagcgtgtgggttggggataagaccaccgccacagacatcaagggcaaggaggtgatggtgttgggagaggtgaacattaacaacagtgtattcaaacagtacttttttgagaccaagtgccgggacccaaatcccgttgacagcgggtgccggggcattgactcaaagcactggaactcatattgtaccacgactcacacctttgtcaaggcgctgaccatggatggcaagcaggctgcctggtggtttatccggatagatacggcctgtgtgtgtgtgctcagcaggaaggctgtgagaagagcctga

SEQ ID NO: 11 - DNA, 735 bp, synthetic construct
  misc_feature 1..735: note = IGK19-NGFmut coding region sequence
  source 1..735: mol_type = other DNA
atggagacagacacactcctgctatgggtactgctgctctgggttccaggttccactggtgacgaaccacactcagagagcaatgtccctgcaggacacaccatcccccaagcccactggactaaacttcagcattcccttgacactgcccttcgcagagcccgcagcgccccggcagcggcgatagctgcacgcgtggcggggcagacccgcaacattactgtggaccccaggctgtttaaaaagcggcgactccgttcaccccgtgtgctgtttagcacccagcctccccgtgaagctgcagacactcaggatctggacttcgaggtcggtggtgctgcccccttcaacaggactcacaggagcaagcggtcatcatcccatcccatcttccacaggggcgaattctcggtgtgtgacagtgtcagcgtgtgggttggggataagaccaccgccacagacatcaagggcaaggaggtgatggtgttgggagaggtgaacattaacaacagtgtattcaaacagtacttttttgagaccaagtgccgggacccaaatcccgttgacagcgggtgccggggcattgactcaaagcactggaactcatattgtaccacgactcacacctttgtcaaggcgctgaccatggatggcaagcaggctgcctggtggtttatccggatagatacggcctgtgtgtgtgtgctcagcaggaaggctgtgagaagagcctga

SEQ ID NO: 12 - DNA, 726 bp, synthetic construct
  misc_feature 1..726: note = BDNF19-NGFmut coding region sequence
  source 1..726: mol_type = other DNA
atgaccatccttttccttactatggttatttcatactttggttgcatgaaggctgaaccacactcagagagcaatgtccctgcaggacacaccatcccccaagcccactggactaaacttcagcattcccttgacactgcccttcgcagagcccgcagcgccccggcagcggcgatagctgcacgcgtggcggggcagacccgcaacattactgtggaccccaggctgtttaaaaagcggcgactccgttcaccccgtgtgctgtttagcacccagcctccccgtgaagctgcagacactcaggatctggacttcgaggtcggtggtgctgcccccttcaacaggactcacaggagcaagcggtcatcatcccatcccatcttccacaggggcgaattctcggtgtgtgacagtgtcagcgtgtgggttggggataagaccaccgccacagacatcaagggcaaggaggtgatggtgttgggagaggtgaacattaacaacagtgtattcaaacagtacttttttgagaccaagtgccgggacccaaatcccgttgacagcgggtgccggggcattgactcaaagcactggaactcatattgtaccacgactcacacctttgtcaaggcgctgaccatggatggcaagcaggctgcctggtggtttatccggatagatacggcctgtgtgtgtgtgctcagcaggaaggctgtgagaagagcctga

SEQ ID NO: 13 - protein, 241 aa, synthetic construct
  REGION 1..241: note = NGFwt amino acid sequence
MSMLFYTLITAFLIGIQAEPHSESNVPAGHTIPQAHWTKLQHSLDTALRRARSAPAAAIAARVAGQTRNITVDPRLFKKRRLRSPRVLFSTQPPREAADTQDLDFEVGGAAPFNRTHRSKRSSSHPIFHRGEFSVCDSVSVWVGDKTTATDIKGKEVMVLGEVNINNSVFKQYFFETKCRDPNPVDSGCRGIDSKHWNSYCTTTHTFVKALTMDGKQAAWRFIRIDTACVCVLSRKAVRRA

SEQ ID NO: 14 - protein, 241 aa, synthetic construct
  REGION 1..241: note = NGFmut amino acid sequence
MSMLFYTLITAFLIGIQAEPHSESNVPAGHTIPQAHWTKLQHSLDTALRRARSAPAAAIAARVAGQTRNITVDPRLFKKRRLRSPRVLFSTQPPREAADTQDLDFEVGGAAPFNRTHRSKRSSSHPIFHRGEFSVCDSVSVWVGDKTTATDIKGKEVMVLGEVNINNSVFKQYFFETKCRDPNPVDSGCRGIDSKHWNSYCTTTHTFVKALTMDGKQAAWWFIRIDTACVCVLSRKAVRRA

SEQ ID NO: 15 - protein, 253 aa, synthetic construct
  REGION 1..253: note = IGK19-NGFmut amino acid sequence
METDTLLLWVLLLWVPGSTGDEPHSESNVPAGHTIPQAHWTKLQHSLDTALRRARSAPAAAIAARVAGQTRNITVDPRLFKKRRLRSPRVLFSTQPPREAADTQDLDFEVGGAAPFNRTHRSKRSSSHPIFHRGEFSVCDSVSVWVGDKTTATDIKGKEVMVLGEVNINNSVFKQYFFETKCRDPNPVDSGCRGIDSKHWNSYCTTTHTFVKALTMDGKQAAWWFIRIDTACVCVLSRKAVRRAYPYDVPDYA

SEQ ID NO: 16 - protein, 141 aa, synthetic construct
  REGION 1..141: note = IGK122-NGFmut amino acid sequence
METDTLLLWVLLLWVPGSTGDSSSHPIFHRGEFSVCDSVSVWVGDKTTATDIKGKEVMVLGEVNINNSVFKQYFFETKCRDPNPVDSGCRGIDSKHWNSYCTTTHTFVKALTMDGKQAAWWFIRIDTACVCVLSRKAVRRA

SEQ ID NO: 17 - protein, 312 aa, synthetic construct
  REGION 1..312: note = IGK19-NGF-PDGFRmut amino acid sequence
METDTLLLWVLLLWVPGSTGDEPHSESNVPAGHTIPQAHWTKLQHSLDTALRRARSAPAAAIAARVAGQTRNITVDPRLFKKRRLRSPRVLFSTQPPREAADTQDLDFEVGGAAPFNRTHRSKRSSSHPIFHRGEFSVCDSVSVWVGDKTTATDIKGKEVMVLGEVNINNSVFKQYFFETKCRDPNPVDSGCRGIDSKHWNSYCTTTHTFVKALTMDGKQAAWWFIRIDTACVCVLSRKAVRRAYPYDVPDYAYPYDVPDYANAVGQDTQEVIVVPHSLPFKVVVISAILALVVLTIISLIILIMLWQKKPR

SEQ ID NO: 18 - protein, 200 aa, synthetic construct
  REGION 1..200: note = IGK122-NGF-PDGFRmut amino acid sequence
METDTLLLWVLLLWVPGSTGDSSSHPIFHRGEFSVCDSVSVWVGDKTTATDIKGKEVMVLGEVNINNSVFKQYFFETKCRDPNPVDSGCRGIDSKHWNSYCTTTHTFVKALTMDGKQAAWWFIRIDTACVCVLSRKAVRRAYPYDVPDYANAVGQDTQEVIVVPHSLPFKVVVISAILALVVLTIISLIILIMLWQKKPR

SEQ ID NO: 19 - protein, 241 aa, synthetic construct
  REGION 1..241: note = BDNF19-NGFmut amino acid sequence
MTILFLTMVISYFGCMKAEPHSESNVPAGHTIPQAHWTKLQHSLDTALRRARSAPAAAIAARVAGQTRNITVDPRLFKKRRLRSPRVLFSTQPPREAADTQDLDFEVGGAAPFNRTHRSKRSSSHPIFHRGEFSVCDSVSVWVGDKTTATDIKGKEVMVLGEVNINNSVFKQYFFETKCRDPNPVDSGCRGIDSKHWNSYCTTTHTFVKALTMDGKQAAWWFIRIDTACVCVLSRKAVRRA

SEQ ID NO: 20 - protein, 248 aa, synthetic construct
  REGION 1..248: note = BDNF122-NGFmut amino acid sequence
MTILFLTMVISYFGCMKAAPMKEANIRGQGGLAYPGVRTHGTLESVNGPKAGSRGLTSLADTFEHVIEELLDEDQKVRPNEENNKDADLYTSRVMLSSQVPLEPPLLFLLEEYKNYLDAANMSMRVRRSSSHPIFHRGEFSVCDSVSVWVGDKTTATDIKGKEVMVLGEVNINNSVFKQYFFETKCRDPNPVDSGCRGIDSKHWNSYCTTTHTFVKALTMDGKQAAWWFIRIDTACVCVLSRKAVRRA

SEQ ID NO: 21 - RNA, 723 nt, synthetic construct
  misc_feature 1..723: note = NGFwt mRNA sequence
  source 1..723: mol_type = other RNA
atgtccatgttgttctacactctgatcacagcttttctgatcggcatacaggcggaaccacactcagagagcaatgtccctgcaggacacaccatcccccaagcccactggactaaacttcagcattcccttgacactgcccttcgcagagcccgcagcgccccggcagcggcgatagctgcacgcgtggcggggcagacccgcaacattactgtggaccccaggctgtttaaaaagcggcgactccgttcaccccgtgtgctgtttagcacccagcctccccgtgaagctgcagacactcaggatctggacttcgaggtcggtggtgctgcccccttcaacaggactcacaggagcaagcggtcatcatcccatcccatcttccacaggggcgaattctcggtgtgtgacagtgtcagcgtgtgggttggggataagaccaccgccacagacatcaagggcaaggaggtgatggtgttgggagaggtgaacattaacaacagtgtattcaaacagtacttttttgagaccaagtgccgggacccaaatcccgttgacagcgggtgccggggcattgactcaaagcactggaactcatattgtaccacgactcacacctttgtcaaggcgctgaccatggatggcaagcaggctgcctggcggtttatccggatagatacggcctgtgtgtgtgtgctcagcaggaaggctgtgagaagagcc

SEQ ID NO: 22 - RNA, 723 nt, synthetic construct
  misc_feature 1..723: note = NGFmut mRNA sequence
  source 1..723: mol_type = other RNA
atgtccatgttgttctacacactgatcaccgccttcctgatcggcatccaggccgagcctcacagcgagtccaatgtgcccgccggccacaccatcccccaggctcattggaccaagctgcagcactccctggatacagccctgagaagagccagatccgcccctgccgccgccatcgctgctagagtggccggacagacaaggaacatcacagtggaccctagactgtttaagaagagaagactgaggagccccagagtgctgttctccacacagccccccagagaggccgccgacacacaggacctggatttcgaggtgggcggcgccgccccttttaacagaacacacagatccaagaggtccagctcccaccctatcttccacagaggcgagttcagcgtgtgcgactccgtgagcgtgtgggtgggcgacaagaccaccgccaccgacatcaagggcaaggaggtcatggtgctgggcgaggtgaacatcaataacagcgtgtttaagcagtactttttcgagaccaagtgcagagaccctaaccctgtggactccggctgtagaggcatcgactccaagcactggaatagctactgcaccacaacccacacattcgtgaaggccctgacaatggacggcaagcaggccgcctggtggttcatcagaatcgacaccgcctgtgtgtgtgtgctgagcagaaaggctgtgagaagagcc

SEQ ID NO: 23 - RNA, 762 nt, synthetic construct
  misc_feature 1..762: note = IGK19-NGFmut mRNA sequence
  source 1..762: mol_type = other RNA
atggagacagacacactcctgctatgggtactgctgctctgggttccaggttccaccggagacgagcctcacagcgagtccaatgtgcccgccggccacaccatcccccaggctcattggaccaagctgcagcactccctggatacagccctgagaagagccagatccgcccctgccgccgccatcgctgctagagtggccggacagacaaggaacatcacagtggaccctagactgtttaagaagagaagactgaggagccccagagtgctgttctccacacagccccccagagaggccgccgacacacaggacctggatttcgaggtgggcggcgccgccccttttaacagaacacacagatccaagaggtccagctcccaccctatcttccacagaggcgagttcagcgtgtgcgactccgtgagcgtgtgggtgggcgacaagaccaccgccaccgacatcaagggcaaggaggtcatggtgctgggcgaggtgaacatcaataacagcgtgtttaagcagtactttttcgagaccaagtgcagagaccctaaccctgtggactccggctgtagaggcatcgactccaagcactggaatagctactgcaccacaacccacacattcgtgaaggccctgacaatggacggcaagcaggccgcctggagattcatcagaatcgacaccgcctgtgtgtgtgtgctgagcagaaaggccgtgagaagggcctacccgtacgacgtgccggactacgcctga

SEQ ID NO: 24 - RNA, 423 nt, synthetic construct
  misc_feature 1..423: note = IGK122-NGFmut mRNA sequence
  source 1..423: mol_type = other RNA
atggagacagacacactcctgctatgggtactgctgctctgggttccaggttccaccggagactccagctcccaccctatcttccacagaggcgagttcagcgtgtgcgactccgtgagcgtgtgggtgggcgacaagaccaccgccaccgacatcaagggcaaggaggtcatggtgctgggcgaggtgaacatcaataacagcgtgtttaagcagtactttttcgagaccaagtgcagagaccctaaccctgtggactccggctgtagaggcatcgactccaagcactggaatagctactgcaccacaacccacacattcgtgaaggccctgacaatggacggcaagcaggccgcctggtggttcatcagaatcgacaccgcctgtgtgtgtgtgctgagcagaaaggctgtgagaagagcc

SEQ ID NO: 25 - RNA, 939 nt, synthetic construct
  misc_feature 1..939: note = IGK19-NGF-PDGFRmut mRNA sequence
  source 1..939: mol_type = other RNA
atggagacagacacactcctgctatgggtactgctgctctgggttccaggttccaccggagacgagcctcacagcgagtccaatgtgcccgccggccacaccatcccccaggctcattggaccaagctgcagcactccctggatacagccctgagaagagccagatccgcccctgccgccgccatcgctgctagagtggccggacagacaaggaacatcacagtggaccctagactgtttaagaagagaagactgaggagccccagagtgctgttctccacacagccccccagagaggccgccgacacacaggacctggatttcgaggtgggcggcgccgccccttttaacagaacacacagatccaagaggtccagctcccaccctatcttccacagaggcgagttcagcgtgtgcgactccgtgagcgtgtgggtgggcgacaagaccaccgccaccgacatcaagggcaaggaggtcatggtgctgggcgaggtgaacatcaataacagcgtgtttaagcagtactttttcgagaccaagtgcagagaccctaaccctgtggactccggctgtagaggcatcgactccaagcactggaatagctactgcaccacaacccacacattcgtgaaggccctgacaatggacggcaagcaggccgcctggagattcatcagaatcgacaccgcctgtgtgtgtgtgctgagcagaaaggccgtgagaagggcctacccgtacgacgtgccggactacgcctgatacccgtacgacgtgccggactacgccaatgctgtgggccaggacacgcaggaggtcatcgtggtgccacactccttgccctttaaggtggtggtgatctcagccatcctggccctggtggtgctcaccatcatctcccttatcatcctcatcatgctttggcagaagaagccacgt

SEQ ID NO: 26 - RNA, 600 nt, synthetic construct
  misc_feature 1..600: note = IGK122-NGF-PDGFRmut mRNA sequence
  source 1..600: mol_type = other RNA
atggagacagacacactcctgctatgggtactgctgctctgggttccaggttccaccggagactccagctcccaccctatcttccacagaggcgagttcagcgtgtgcgactccgtgagcgtgtgggtgggcgacaagaccaccgccaccgacatcaagggcaaggaggtcatggtgctgggcgaggtgaacatcaataacagcgtgtttaagcagtactttttcgagaccaagtgcagagaccctaaccctgtggactccggctgtagaggcatcgactccaagcactggaatagctactgcaccacaacccacacattcgtgaaggccctgacaatggacggcaagcaggccgcctggtggttcatcagaatcgacaccgcctgtgtgtgtgtgctgagcagaaaggctgtgagaagagcctacccgtacgacgtgccggactacgccaatgctgtgggccaggacacgcaggaggtcatcgtggtgccacactccttgccctttaaggtggtggtgatctcagccatcctggccctggtggtgctcaccatcatctcccttatcatcctcatcatgctttggcagaagaagccacgt

SEQ ID NO: 27 - RNA, 723 nt, synthetic construct
  misc_feature 1..723: note = BDNF19-NGFmut mRNA sequence
  source 1..723: mol_type = other RNA
atgaccatcctgttcctgacaatggtcattagctacttcggctgcatgaaggccgagcctcacagcgagtccaatgtgcccgccggccacaccatcccccaggctcattggaccaagctgcagcactccctggatacagccctgagaagagccagatccgcccctgccgccgccatcgctgctagagtggccggacagacaaggaacatcacagtggaccctagactgtttaagaagagaagactgaggagccccagagtgctgttctccacacagccccccagagaggccgccgacacacaggacctggatttcgaggtgggcggcgccgccccttttaacagaacacacagatccaagaggtccagctcccaccctatcttccacagaggcgagttcagcgtgtgcgactccgtgagcgtgtgggtgggcgacaagaccaccgccaccgacatcaagggcaaggaggtcatggtgctgggcgaggtgaacatcaataacagcgtgtttaagcagtactttttcgagaccaagtgcagagaccctaaccctgtggactccggctgtagaggcatcgactccaagcactggaatagctactgcaccacaacccacacattcgtgaaggccctgacaatggacggcaagcaggccgcctggtggttcatcagaatcgacaccgcctgtgtgtgtgtgctgagcagaaaggctgtgagaagagcc

SEQ ID NO: 28 - RNA, 744 nt, synthetic construct
  misc_feature 1..744: note = BDNF122-NGFmut mRNA sequence
  source 1..744: mol_type = other RNA
atgaccatcctgttcctgacaatggtcattagctacttcggctgcatgaaggccgcccccatgaaggaggccaacatcagaggccagggcggcctggcctaccccggagtgagaacacacggcacactggagtccgtgaacggccccaaggccggctccaggggactgacaagcctggccgataccttcgagcacgtgatcgaggagctgctggacgaggaccagaaggtgaggcccaatgaggagaataataaggacgccgacctgtacacctccagggtcatgctgagcagccaggtgcccctggagcccccactgctgttcctgctggaggagtacaagaattacctggacgccgccaatatgtccatgagagtgagaaggtccagctcccaccctatcttccacagaggcgagttcagcgtgtgcgactccgtgagcgtgtgggtgggcgacaagaccaccgccaccgacatcaagggcaaggaggtcatggtgctgggcgaggtgaacatcaataacagcgtgtttaagcagtactttttcgagaccaagtgcagagaccctaaccctgtggactccggctgtagaggcatcgactccaagcactggaatagctactgcaccacaacccacacattcgtgaaggccctgacaatggacggcaagcaggccgcctggtggttcatcagaatcgacaccgcctgtgtgtgtgtgctgagcagaaaggctgtgagaagagcc

SEQ ID NO: 29 - protein, 18 aa, synthetic construct
  REGION 1..18: note = NGF signal peptide
MSMLFYTLITAFLIGIQA

SEQ ID NO: 30 - protein, 21 aa, synthetic construct
  REGION 1..21: note = IGK signaling peptide
METDTLLLWVLLLWVPGSTGD

SEQ ID NO: 31 - protein, 18 aa, synthetic construct
  REGION 1..18: note = BDNF signaling peptide
MTILFLTMVISYFGCMKA

SEQ ID NO: 32 - protein, 120 aa, synthetic construct
  REGION 1..120: note = Matured NGFwt
SSSHPIFHRGEFSVCDSVSVWVGDKTTATDIKGKEVMVLGEVNINNSVFKQYFFETKCRDPNPVDSGCRGIDSKHWNSYCTTTHTFVKALTMDGKQAAWRFIRIDTACVCVLSRKAVRRA

SEQ ID NO: 33 - protein, 120 aa, synthetic construct
  REGION 1..120: note = Matured NGFmut
SSSHPIFHRGEFSVCDSVSVWVGDKTTATDIKGKEVMVLGEVNINNSVFKQYFFETKCRDPNPVDSGCRGIDSKHWNSYCTTTHTFVKALTMDGKQAAWWFIRIDTACVCVLSRKAVRRA

SEQ ID NO: 34 - protein, 103 aa, synthetic construct
  REGION 1..103: note = Leading peptide
EPHSESNVPAGHTIPQAHWTKLQHSLDTALRRARSAPAAAIAARVAGQTRNITVDPRLFKKRRLRSPRVLFSTQPPREAADTQDLDFEVGGAAPFNRTHRSKR

SEQ ID NO: 35 - protein, 20 aa, synthetic construct
  REGION 1..20: note = Human IL-2 signal peptide
MYRMQLLSCIALSLALVTNS

SEQ ID NO: 36 - protein, 19 aa, synthetic construct
  REGION 1..19: note = Azurin preprotein signal peptide
MTRLTVLALLAGLLASSRA

SEQ ID NO: 37 - protein, 19 aa, synthetic construct
  REGION 1..19: note = Immunoglobulin heavy chain signal peptide
MDWTWRVFCLLAVTPGAHP

SEQ ID NO: 38 - protein, 20 aa, synthetic construct
  REGION 1..20: note = Cystatin-S precursor signaling peptide
MARPLCTLLLLMATLAGALA

SEQ ID NO: 39 - protein, 38 aa, synthetic construct
  REGION 1..38: note = Gp67 signal peptide
MLLVNQSHQGFNKEHTSKMVSAIVLYVLLAAAAHSAFA

SEQ ID NO: 40 - protein, 21 aa, synthetic construct
  REGION 1..21: note = HBM signal peptides
MKFLVNVALVFMVVYISYIYA

SEQ ID NO: 41 - protein, 20 aa, synthetic construct
  REGION 1..20: note = Gp64 signal peptide
MVSAIVLYVLLAAAAHSAFA

SEQ ID NO: 42 - protein, 18 aa, synthetic construct
  REGION 1..18: note = Albumin signaling peptide
MKWVTFISLLFLFSSAYS

SEQ ID NO: 43 - protein, 26 aa, synthetic construct
  REGION 1..26: note = SP signal peptide
MRVTAPRTLILLLSGALALTETWAGS

SEQ ID NO: 44 - DNA, 1431 bp, synthetic construct
  misc_feature 1..1431: note = NGFwt-Fc1 optimized coding region sequence
  source 1..1431: mol_type = other DNA
atgtccatgttgttctacacactgatcaccgccttcctgatcggcatccaggccgagcctcacagcgagtccaatgtgcccgccggccacaccatcccccaggctcattggaccaagctgcagcactccctggatacagccctgagaagagccagatccgcccctgccgccgccatcgctgctagagtggccggacagacaaggaacatcacagtggaccctagactgtttaagaagagaagactgaggagccccagagtgctgttctccacacagccccccagagaggccgccgacacacaggacctggatttcgaggtgggcggcgccgccccttttaacagaacacacagatccaagaggtccagctcccaccctatcttccacagaggcgagttcagcgtgtgcgactccgtgagcgtgtgggtgggcgacaagaccaccgccaccgacatcaagggcaaggaggtcatggtgctgggcgaggtgaacatcaataacagcgtgtttaagcagtactttttcgagaccaagtgcagagaccctaaccctgtggactccggctgtagaggcatcgactccaagcactggaatagctactgcaccacaacccacacattcgtgaaggccctgacaatggacggcaagcaggccgcctggagattcatcagaatcgacaccgcctgtgtgtgtgtgctgagcagaaaggctgtgagaagagccggaagcggatctgagcccaagagccaggacaagacccacacctgccctccctgtcctgcccccgagctgctgggaggaccttccgtgttcctgttcccccctaagcctaaggacaccctgatgatcagcaggacccctgaggtgacctgtgtggtggtggatgtgtcccacgaggaccctgaggtgaagttcaactggtatgtggacggcgtggaggtgcacaatgctaagaccaagcccagggaagagcagtacaacagcacctatagggtggtgagcgtgctgaccgtgctgcaccaggattggctgaatggcaaggagtacaagtgtaaggtgagcaacaaggctctgcccgctcctatcgagaagaccatctccaaggccaagggccagcccagggagcctcaggtgtataccctgcccccttccagggatgagctgaccaagaatcaggtgtccctgacctgtctggtgaagggcttttacccctccgacatcgctgtggagtgggagagcaatggccagcctgagaacaactacaagaccacccctcccgtgctggattccgacggctcctttttcctgtatagcaagctgaccgtggacaagtcccggtggcagcagggcaacgtgttttcctgtagcgtgatgcacgaggccctgcacaaccactacacccagaagtccctgtccctgtcccctggcaag

SEQ ID NO: 45 - DNA, 1428 bp, synthetic construct
  misc_feature 1..1428: note = NGFwt-Fc2 optimized coding region sequence
  source 1..1428: mol_type = other DNA
atgtccatgttgttctacacactgatcaccgccttcctgatcggcatccaggccgagcctcacagcgagtccaatgtgcccgccggccacaccatcccccaggctcattggaccaagctgcagcactccctggatacagccctgagaagagccagatccgcccctgccgccgccatcgctgctagagtggccggacagacaaggaacatcacagtggaccctagactgtttaagaagagaagactgaggagccccagagtgctgttctccacacagccccccagagaggccgccgacacacaggacctggatttcgaggtgggcggcgccgccccttttaacagaacacacagatccaagaggtccagctcccaccctatcttccacagaggcgagttcagcgtgtgcgactccgtgagcgtgtgggtgggcgacaagaccaccgccaccgacatcaagggcaaggaggtcatggtgctgggcgaggtgaacatcaataacagcgtgtttaagcagtactttttcgagaccaagtgcagagaccctaaccctgtggactccggctgtagaggcatcgactccaagcactggaatagctactgcaccacaacccacacattcgtgaaggccctgacaatggacggcaagcaggccgcctggagattcatcagaatcgacaccgcctgtgtgtgtgtgctgagcagaaaggctgtgagaagagccggatctggcagcgataagaagatcgtgcccagggattgcggctgcaagccttgcatctgcaccgtgcccgaggtgtccagcgtgttcatcttcccccctaagcccaaggatgtgctgaccatcaccctgacccccaaggtgacctgtgtggtggtggctatcagcaaggatgaccccgaggtgcagtttagctggtttgtggatgatgtggaggtgcacaccgcccagacccagcccagagaggagcagtttaattccacctttcggtccgtgtccgagctgcctatcatgcaccaggattggctgaacggcaaggagttcaagtgcagggtgaacagcgctgctttccccgcccccatcgagaagaccatcagcaagaccaagggcaggcccaaggcccctcaggtgtacaccatccccccccccaaggagcagatggccaaggataaggtgagcctgacctgcatgatcaccgatttcttccctgaggatatcaccgtggagtggcagtggaatggccagcccgccgagaattacaagaatacccagcccatcatggacaccgacggcagctatttcgtgtattccaagctgaatgtgcagaagtccaattgggaggccggcaacaccttcacctgcagcgtgctgcacgagggcctgcacaatcaccacaccgagaagagcctgtcccactcccccggcaag

SEQ ID NO: 46 - DNA, 1440 bp, synthetic construct
  misc_feature 1..1440: note = IGK19-NGFmut-Fc1 optimized sequence of the coding region
  source 1..1440: mol_type = other DNA
atggagacagacacactcctgctatgggtactgctgctctgggttccaggttccaccggagacgagcctcacagcgagtccaatgtgcccgccggccacaccatcccccaggctcattggaccaagctgcagcactccctggatacagccctgagaagagccagatccgcccctgccgccgccatcgctgctagagtggccggacagacaaggaacatcacagtggaccctagactgtttaagaagagaagactgaggagccccagagtgctgttctccacacagccccccagagaggccgccgacacacaggacctggatttcgaggtgggcggcgccgccccttttaacagaacacacagatccaagaggtccagctcccaccctatcttccacagaggcgagttcagcgtgtgcgactccgtgagcgtgtgggtgggcgacaagaccaccgccaccgacatcaagggcaaggaggtcatggtgctgggcgaggtgaacatcaataacagcgtgtttaagcagtactttttcgagaccaagtgcagagaccctaaccctgtggactccggctgtagaggcatcgactccaagcactggaatagctactgcaccacaacccacacattcgtgaaggccctgacaatggacggcaagcaggccgcctggtggttcatcagaatcgacaccgcctgtgtgtgtgtgctgagcagaaaggctgtgagaagagccggaagcggatctgagcccaagagccaggacaagacccacacctgccctccctgtcctgcccccgagctgctgggaggaccttccgtgttcctgttcccccctaagcctaaggacaccctgatgatcagcaggacccctgaggtgacctgtgtggtggtggatgtgtcccacgaggaccctgaggtgaagttcaactggtatgtggacggcgtggaggtgcacaatgctaagaccaagcccagggaagagcagtacaacagcacctatagggtggtgagcgtgctgaccgtgctgcaccaggattggctgaatggcaaggagtacaagtgtaaggtgagcaacaaggctctgcccgctcctatcgagaagaccatctccaaggccaagggccagcccagggagcctcaggtgtataccctgcccccttccagggatgagctgaccaagaatcaggtgtccctgacctgtctggtgaagggcttttacccctccgacatcgctgtggagtgggagagcaatggccagcctgagaacaactacaagaccacccctcccgtgctggattccgacggctcctttttcctgtatagcaagctgaccgtggacaagtcccggtggcagcagggcaacgtgttttcctgtagcgtgatgcacgaggccctgcacaaccactacacccagaagtccctgtccctgtcccctggcaag

SEQ ID NO: 47 - DNA, 1437 bp, synthetic construct
  misc_feature 1..1437: note = IGK19-NGFmut-Fc2 optimized sequence of the coding region
  source 1..1437: mol_type = other DNA
atggagacagacacactcctgctatgggtactgctgctctgggttccaggttccaccggagacgagcctcacagcgagtccaatgtgcccgccggccacaccatcccccaggctcattggaccaagctgcagcactccctggatacagccctgagaagagccagatccgcccctgccgccgccatcgctgctagagtggccggacagacaaggaacatcacagtggaccctagactgtttaagaagagaagactgaggagccccagagtgctgttctccacacagccccccagagaggccgccgacacacaggacctggatttcgaggtgggcggcgccgccccttttaacagaacacacagatccaagaggtccagctcccaccctatcttccacagaggcgagttcagcgtgtgcgactccgtgagcgtgtgggtgggcgacaagaccaccgccaccgacatcaagggcaaggaggtcatggtgctgggcgaggtgaacatcaataacagcgtgtttaagcagtactttttcgagaccaagtgcagagaccctaaccctgtggactccggctgtagaggcatcgactccaagcactggaatagctactgcaccacaacccacacattcgtgaaggccctgacaatggacggcaagcaggccgcctggtggttcatcagaatcgacaccgcctgtgtgtgtgtgctgagcagaaaggctgtgagaagagccggatctggcagcgataagaagatcgtgcccagggattgcggctgcaagccttgcatctgcaccgtgcccgaggtgtccagcgtgttcatcttcccccctaagcccaaggatgtgctgaccatcaccctgacccccaaggtgacctgtgtggtggtggctatcagcaaggatgaccccgaggtgcagtttagctggtttgtggatgatgtggaggtgcacaccgcccagacccagcccagagaggagcagtttaattccacctttcggtccgtgtccgagctgcctatcatgcaccaggattggctgaacggcaaggagttcaagtgcagggtgaacagcgctgctttccccgcccccatcgagaagaccatcagcaagaccaagggcaggcccaaggcccctcaggtgtacaccatccccccccccaaggagcagatggccaaggataaggtgagcctgacctgcatgatcaccgatttcttccctgaggatatcaccgtggagtggcagtggaatggccagcccgccgagaattacaagaatacccagcccatcatggacaccgacggcagctatttcgtgtattccaagctgaatgtgcagaagtccaattgggaggccggcaacaccttcacctgcagcgtgctgcacgagggcctgcacaatcaccacaccgagaagagcctgtcccactcccccggcaag

SEQ ID NO: 48 - RNA, 1431 nt, synthetic construct
  misc_feature 1..1431: note = NGFwt-Fc1 mRNA Sequence
  source 1..1431: mol_type = other RNA
atgtccatgttgttctacacactgatcaccgccttcctgatcggcatccaggccgagcctcacagcgagtccaatgtgcccgccggccacaccatcccccaggctcattggaccaagctgcagcactccctggatacagccctgagaagagccagatccgcccctgccgccgccatcgctgctagagtggccggacagacaaggaacatcacagtggaccctagactgtttaagaagagaagactgaggagccccagagtgctgttctccacacagccccccagagaggccgccgacacacaggacctggatttcgaggtgggcggcgccgccccttttaacagaacacacagatccaagaggtccagctcccaccctatcttccacagaggcgagttcagcgtgtgcgactccgtgagcgtgtgggtgggcgacaagaccaccgccaccgacatcaagggcaaggaggtcatggtgctgggcgaggtgaacatcaataacagcgtgtttaagcagtactttttcgagaccaagtgcagagaccctaaccctgtggactccggctgtagaggcatcgactccaagcactggaatagctactgcaccacaacccacacattcgtgaaggccctgacaatggacggcaagcaggccgcctggagattcatcagaatcgacaccgcctgtgtgtgtgtgctgagcagaaaggctgtgagaagagccggaagcggatctgagcccaagagccaggacaagacccacacctgccctccctgtcctgcccccgagctgctgggaggaccttccgtgttcctgttcccccctaagcctaaggacaccctgatgatcagcaggacccctgaggtgacctgtgtggtggtggatgtgtcccacgaggaccctgaggtgaagttcaactggtatgtggacggcgtggaggtgcacaatgctaagaccaagcccagggaagagcagtacaacagcacctatagggtggtgagcgtgctgaccgtgctgcaccaggattggctgaatggcaaggagtacaagtgtaaggtgagcaacaaggctctgcccgctcctatcgagaagaccatctccaaggccaagggccagcccagggagcctcaggtgtataccctgcccccttccagggatgagctgaccaagaatcaggtgtccctgacctgtctggtgaagggcttttacccctccgacatcgctgtggagtgggagagcaatggccagcctgagaacaactacaagaccacccctcccgtgctggattccgacggctcctttttcctgtatagcaagctgaccgtggacaagtcccggtggcagcagggcaacgtgttttcctgtagcgtgatgcacgaggccctgcacaaccactacacccagaagtccctgtccctgtcccctggcaag

SEQ ID NO: 49 - RNA, 1428 nt, synthetic construct
  misc_feature 1..1428: note = NGFwt-Fc2 mRNA sequences
  source 1..1428: mol_type = other RNA
atgtccatgttgttctacacactgatcaccgccttcctgatcggcatccaggccgagcctcacagcgagtccaatgtgcccgccggccacaccatcccccaggctcattggaccaagctgcagcactccctggatacagccctgagaagagccagatccgcccctgccgccgccatcgctgctagagtggccggacagacaaggaacatcacagtggaccctagactgtttaagaagagaagactgaggagccccagagtgctgttctccacacagccccccagagaggccgccgacacacaggacctggatttcgaggtgggcggcgccgccccttttaacagaacacacagatccaagaggtccagctcccaccctatcttccacagaggcgagttcagcgtgtgcgactccgtgagcgtgtgggtgggcgacaagaccaccgccaccgacatcaagggcaaggaggtcatggtgctgggcgaggtgaacatcaataacagcgtgtttaagcagtactttttcgagaccaagtgcagagaccctaaccctgtggactccggctgtagaggcatcgactccaagcactggaatagctactgcaccacaacccacacattcgtgaaggccctgacaatggacggcaagcaggccgcctggagattcatcagaatcgacaccgcctgtgtgtgtgtgctgagcagaaaggctgtgagaagagccggatctggcagcgataagaagatcgtgcccagggattgcggctgcaagccttgcatctgcaccgtgcccgaggtgtccagcgtgttcatcttcccccctaagcccaaggatgtgctgaccatcaccctgacccccaaggtgacctgtgtggtggtggctatcagcaaggatgaccccgaggtgcagtttagctggtttgtggatgatgtggaggtgcacaccgcccagacccagcccagagaggagcagtttaattccacctttcggtccgtgtccgagctgcctatcatgcaccaggattggctgaacggcaaggagttcaagtgcagggtgaacagcgctgctttccccgcccccatcgagaagaccatcagcaagaccaagggcaggcccaaggcccctcaggtgtacaccatccccccccccaaggagcagatggccaaggataaggtgagcctgacctgcatgatcaccgatttcttccctgaggatatcaccgtggagtggcagtggaatggccagcccgccgagaattacaagaatacccagcccatcatggacaccgacggcagctatttcgtgtattccaagctgaatgtgcagaagtccaattgggaggccggcaacaccttcacctgcagcgtgctgcacgagggcctgcacaatcaccacaccgagaagagcctgtcccactcccccggcaag

SEQ ID NO: 50 - RNA, 1440 nt, synthetic construct
  misc_feature 1..1440: note = IGK19-NGFmut-Fc1 mRNA Sequence
  source 1..1440: mol_type = other RNA
atggagacagacacactcctgctatgggtactgctgctctgggttccaggttccaccggagacgagcctcacagcgagtccaatgtgcccgccggccacaccatcccccaggctcattggaccaagctgcagcactccctggatacagccctgagaagagccagatccgcccctgccgccgccatcgctgctagagtggccggacagacaaggaacatcacagtggaccctagactgtttaagaagagaagactgaggagccccagagtgctgttctccacacagccccccagagaggccgccgacacacaggacctggatttcgaggtgggcggcgccgccccttttaacagaacacacagatccaagaggtccagctcccaccctatcttccacagaggcgagttcagcgtgtgcgactccgtgagcgtgtgggtgggcgacaagaccaccgccaccgacatcaagggcaaggaggtcatggtgctgggcgaggtgaacatcaataacagcgtgtttaagcagtactttttcgagaccaagtgcagagaccctaaccctgtggactccggctgtagaggcatcgactccaagcactggaatagctactgcaccacaacccacacattcgtgaaggccctgacaatggacggcaagcaggccgcctggtggttcatcagaatcgacaccgcctgtgtgtgtgtgctgagcagaaaggctgtgagaagagccggaagcggatctgagcccaagagccaggacaagacccacacctgccctccctgtcctgcccccgagctgctgggaggaccttccgtgttcctgttcccccctaagcctaaggacaccctgatgatcagcaggacccctgaggtgacctgtgtggtggtggatgtgtcccacgaggaccctgaggtgaagttcaactggtatgtggacggcgtggaggtgcacaatgctaagaccaagcccagggaagagcagtacaacagcacctatagggtggtgagcgtgctgaccgtgctgcaccaggattggctgaatggcaaggagtacaagtgtaaggtgagcaacaaggctctgcccgctcctatcgagaagaccatctccaaggccaagggccagcccagggagcctcaggtgtataccctgcccccttccagggatgagctgaccaagaatcaggtgtccctgacctgtctggtgaagggcttttacccctccgacatcgctgtggagtgggagagcaatggccagcctgagaacaactacaagaccacccctcccgtgctggattccgacggctcctttttcctgtatagcaagctgaccgtggacaagtcccggtggcagcagggcaacgtgttttcctgtagcgtgatgcacgaggccctgcacaaccactacacccagaagtccctgtccctgtcccctggcaag

SEQ ID NO: 51 - RNA, 1437 nt, synthetic construct
  misc_feature 1..1437: note = IGK19-NGFmut-Fc2 mRNA Sequence
  source 1..1437: mol_type = other RNA
atggagacagacacactcctgctatgggtactgctgctctgggttccaggttccaccggagacgagcctcacagcgagtccaatgtgcccgccggccacaccatcccccaggctcattggaccaagctgcagcactccctggatacagccctgagaagagccagatccgcccctgccgccgccatcgctgctagagtggccggacagacaaggaacatcacagtggaccctagactgtttaagaagagaagactgaggagccccagagtgctgttctccacacagccccccagagaggccgccgacacacaggacctggatttcgaggtgggcggcgccgccccttttaacagaacacacagatccaagaggtccagctcccaccctatcttccacagaggcgagttcagcgtgtgcgactccgtgagcgtgtgggtgggcgacaagaccaccgccaccgacatcaagggcaaggaggtcatggtgctgggcgaggtgaacatcaataacagcgtgtttaagcagtactttttcgagaccaagtgcagagaccctaaccctgtggactccggctgtagaggcatcgactccaagcactggaatagctactgcaccacaacccacacattcgtgaaggccctgacaatggacggcaagcaggccgcctggtggttcatcagaatcgacaccgcctgtgtgtgtgtgctgagcagaaaggctgtgagaagagccggatctggcagcgataagaagatcgtgcccagggattgcggctgcaagccttgcatctgcaccgtgcccgaggtgtccagcgtgttcatcttcccccctaagcccaaggatgtgctgaccatcaccctgacccccaaggtgacctgtgtggtggtggctatcagcaaggatgaccccgaggtgcagtttagctggtttgtggatgatgtggaggtgcacaccgcccagacccagcccagagaggagcagtttaattccacctttcggtccgtgtccgagctgcctatcatgcaccaggattggctgaacggcaaggagttcaagtgcagggtgaacagcgctgctttccccgcccccatcgagaagaccatcagcaagaccaagggcaggcccaaggcccctcaggtgtacaccatccccccccccaaggagcagatggccaaggataaggtgagcctgacctgcatgatcaccgatttcttccctgaggatatcaccgtggagtggcagtggaatggccagcccgccgagaattacaagaatacccagcccatcatggacaccgacggcagctatttcgtgtattccaagctgaatgtgcagaagtccaattgggaggccggcaacaccttcacctgcagcgtgctgcacgagggcctgcacaatcaccacaccgagaagagcctgtcccactcccccggcaag

SEQ ID NO: 52 - protein, 477 aa, synthetic construct
  REGION 1..477: note = NGFwt-Fc1 amino acid sequence
MSMLFYTLITAFLIGIQAEPHSESNVPAGHTIPQAHWTKLQHSLDTALRRARSAPAAAIAARVAGQTRNITVDPRLFKKRRLRSPRVLFSTQPPREAADTQDLDFEVGGAAPFNRTHRSKRSSSHPIFHRGEFSVCDSVSVWVGDKTTATDIKGKEVMVLGEVNINNSVFKQYFFETKCRDPNPVDSGCRGIDSKHWNSYCTTTHTFVKALTMDGKQAAWRFIRIDTACVCVLSRKAVRRAGSGSEPKSQDKTHTCPPCPAPELLGGPSVFLFPPKPKDTLMISRTPEVTCVVVDVSHEDPEVKFNWYVDGVEVHNAKTKPREEQYNSTYRVVSVLTVLHQDWLNGKEYKCKVSNKALPAPIEKTISKAKGQPREPQVYTLPPSRDELTKNQVSLTCLVKGFYPSDIAVEWESNGQPENNYKTTPPVLDSDGSFFLYSKLTVDKSRWQQGNVFSCSVMHEALHNHYTQKSLSLSPGK

SEQ ID NO: 53 - protein, 476 aa, synthetic construct
  REGION 1..476: note = NGFwt-Fc2 amino acid sequence
MSMLFYTLITAFLIGIQAEPHSESNVPAGHTIPQAHWTKLQHSLDTALRRARSAPAAAIAARVAGQTRNITVDPRLFKKRRLRSPRVLFSTQPPREAADTQDLDFEVGGAAPFNRTHRSKRSSSHPIFHRGEFSVCDSVSVWVGDKTTATDIKGKEVMVLGEVNINNSVFKQYFFETKCRDPNPVDSGCRGIDSKHWNSYCTTTHTFVKALTMDGKQAAWRFIRIDTACVCVLSRKAVRRAGSGSDKKIVPRDCGCKPCICTVPEVSSVFIFPPKPKDVLTITLTPKVTCVVVAISKDDPEVQFSWFVDDVEVHTAQTQPREEQFNSTFRSVSELPIMHQDWLNGKEFKCRVNSAAFPAPIEKTISKTKGRPKAPQVYTIPPPKEQMAKDKVSLTCMITDFFPEDITVEWQWNGQPAENYKNTQPIMDTDGSYFVYSKLNVQKSNWEAGNTFTCSVLHEGLHNHHTEKSLSHSPGK

SEQ ID NO: 54 - protein, 480 aa, synthetic construct
  REGION 1..480: note = IGK19-NGFmut-Fc1 amino acid sequence
METDTLLLWVLLLWVPGSTGDEPHSESNVPAGHTIPQAHWTKLQHSLDTALRRARSAPAAAIAARVAGQTRNITVDPRLFKKRRLRSPRVLFSTQPPREAADTQDLDFEVGGAAPFNRTHRSKRSSSHPIFHRGEFSVCDSVSVWVGDKTTATDIKGKEVMVLGEVNINNSVFKQYFFETKCRDPNPVDSGCRGIDSKHWNSYCTTTHTFVKALTMDGKQAAWWFIRIDTACVCVLSRKAVRRAGSGSEPKSQDKTHTCPPCPAPELLGGPSVFLFPPKPKDTLMISRTPEVTCVVVDVSHEDPEVKFNWYVDGVEVHNAKTKPREEQYNSTYRVVSVLTVLHQDWLNGKEYKCKVSNKALPAPIEKTISKAKGQPREPQVYTLPPSRDELTKNQVSLTCLVKGFYPSDIAVEWESNGQPENNYKTTPPVLDSDGSFFLYSKLTVDKSRWQQGNVFSCSVMHEALHNHYTQKSLSLSPGK

SEQ ID NO: 55 - protein, 479 aa, synthetic construct
  REGION 1..479: note = IGK19-NGFmut-Fc2 amino acid sequence
METDTLLLWVLLLWVPGSTGDEPHSESNVPAGHTIPQAHWTKLQHSLDTALRRARSAPAAAIAARVAGQTRNITVDPRLFKKRRLRSPRVLFSTQPPREAADTQDLDFEVGGAAPFNRTHRSKRSSSHPIFHRGEFSVCDSVSVWVGDKTTATDIKGKEVMVLGEVNINNSVFKQYFFETKCRDPNPVDSGCRGIDSKHWNSYCTTTHTFVKALTMDGKQAAWWFIRIDTACVCVLSRKAVRRAGSGSDKKIVPRDCGCKPCICTVPEVSSVFIFPPKPKDVLTITLTPKVTCVVVAISKDDPEVQFSWFVDDVEVHTAQTQPREEQFNSTFRSVSELPIMHQDWLNGKEFKCRVNSAAFPAPIEKTISKTKGRPKAPQVYTIPPPKEQMAKDKVSLTCMITDFFPEDITVEWQWNGQPAENYKNTQPIMDTDGSYFVYSKLNVQKSNWEAGNTFTCSVLHEGLHNHHTEKSLSHSPGK

SEQ ID NO: 56 - protein, 232 aa, synthetic construct
  REGION 1..232: note = Human Fc-1 amino acid sequence
EPKSQDKTHTCPPCPAPELLGGPSVFLFPPKPKDTLMISRTPEVTCVVVDVSHEDPEVKFNWYVDGVEVHNAKTKPREEQYNSTYRVVSVLTVLHQDWLNGKEYKCKVSNKALPAPIEKTISKAKGQPREPQVYTLPPSRDELTKNQVSLTCLVKGFYPSDIAVEWESNGQPENNYKTTPPVLDSDGSFFLYSKLTVDKSRWQQGNVFSCSVMHEALHNHYTQKSLSLSPGK

SEQ ID NO: 57 - protein, 231 aa, synthetic construct
  REGION 1..231: note = Mouse Fc-2 amino acid sequence
DKKIVPRDCGCKPCICTVPEVSSVFIFPPKPKDVLTITLTPKVTCVVVAISKDDPEVQFSWFVDDVEVHTAQTQPREEQFNSTFRSVSELPIMHQDWLNGKEFKCRVNSAAFPAPIEKTISKTKGRPKAPQVYTIPPPKEQMAKDKVSLTCMITDFFPEDITVEWQWNGQPAENYKNTQPIMDTDGSYFVYSKLNVQKSNWEAGNTFTCSVLHEGLHNHHTEKSLSHSPGK

SEQ ID NO: 58 - protein, 249 aa, synthetic construct
  REGION 1..249: note = SP-19-NGFmut amino acid sequence
MRVTAPRTLILLLSGALALTETWAGSEPHSESNVPAGHTIPQAHWTKLQHSLDTALRRARSAPAAAIAARVAGQTRNITVDPRLFKKRRLRSPRVLFSTQPPREAADTQDLDFEVGGAAPFNRTHRSKRSSSHPIFHRGEFSVCDSVSVWVGDKTTATDIKGKEVMVLGEVNINNSVFKQYFFETKCRDPNPVDSGCRGIDSKHWNSYCTTTHTFVKALTMDGKQAAWWFIRIDTACVCVLSRKAVRRA

SEQ ID NO: 59 - protein, 243 aa, synthetic construct
  REGION 1..243: note = hIL12-19-NGFmut amino acid sequence
MYRMQLLSCIALSLALVTNSEPHSESNVPAGHTIPQAHWTKLQHSLDTALRRARSAPAAAIAARVAGQTRNITVDPRLFKKRRLRSPRVLFSTQPPREAADTQDLDFEVGGAAPFNRTHRSKRSSSHPIFHRGEFSVCDSVSVWVGDKTTATDIKGKEVMVLGEVNINNSVFKQYFFETKCRDPNPVDSGCRGIDSKHWNSYCTTTHTFVKALTMDGKQAAWWFIRIDTACVCVLSRKAVRRA

SEQ ID NO: 60 - protein, 243 aa, synthetic construct
  REGION 1..243: note = Cystatin 19-NGFmut amino acid sequence
MARPLCTLLLLMATLAGALAEPHSESNVPAGHTIPQAHWTKLQHSLDTALRRARSAPAAAIAARVAGQTRNITVDPRLFKKRRLRSPRVLFSTQPPREAADTQDLDFEVGGAAPFNRTHRSKRSSSHPIFHRGEFSVCDSVSVWVGDKTTATDIKGKEVMVLGEVNINNSVFKQYFFETKCRDPNPVDSGCRGIDSKHWNSYCTTTHTFVKALTMDGKQAAWWFIRIDTACVCVLSRKAVRRA

SEQ ID NO: 61 - protein, 242 aa, synthetic construct
  REGION 1..242: note = APP-19-NGFmut amino acid sequence
MTRLTVLALLAGLLASSRAEPHSESNVPAGHTIPQAHWTKLQHSLDTALRRARSAPAAAIAARVAGQTRNITVDPRLFKKRRLRSPRVLFSTQPPREAADTQDLDFEVGGAAPFNRTHRSKRSSSHPIFHRGEFSVCDSVSVWVGDKTTATDIKGKEVMVLGEVNINNSVFKQYFFETKCRDPNPVDSGCRGIDSKHWNSYCTTTHTFVKALTMDGKQAAWWFIRIDTACVCVLSRKAVRRA

SEQ ID NO: 62 - protein, 242 aa, synthetic construct
  REGION 1..242: note = HC-19-NGFmut amino acid sequence
MDWTWRVFCLLAVTPGAHPEPHSESNVPAGHTIPQAHWTKLQHSLDTALRRARSAPAAAIAARVAGQTRNITVDPRLFKKRRLRSPRVLFSTQPPREAADTQDLDFEVGGAAPFNRTHRSKRSSSHPIFHRGEFSVCDSVSVWVGDKTTATDIKGKEVMVLGEVNINNSVFKQYFFETKCRDPNPVDSGCRGIDSKHWNSYCTTTHTFVKALTMDGKQAAWWFIRIDTACVCVLSRKAVRRA

SEQ ID NO: 63 - protein, 261 aa, synthetic construct
  REGION 1..261: note = Gp67-19-NGFmut amino acid sequence
MLLVNQSHQGFNKEHTSKMVSAIVLYVLLAAAAHSAFAEPHSESNVPAGHTIPQAHWTKLQHSLDTALRRARSAPAAAIAARVAGQTRNITVDPRLFKKRRLRSPRVLFSTQPPREAADTQDLDFEVGGAAPFNRTHRSKRSSSHPIFHRGEFSVCDSVSVWVGDKTTATDIKGKEVMVLGEVNINNSVFKQYFFETKCRDPNPVDSGCRGIDSKHWNSYCTTTHTFVKALTMDGKQAAWWFIRIDTACVCVLSRKAVRRA

SEQ ID NO: 64 - protein, 244 aa, synthetic construct
  REGION 1..244: note = Amino acid sequence of HBM-19-NGFmut
MKFLVNVALVFMVVYISYIYAEPHSESNVPAGHTIPQAHWTKLQHSLDTALRRARSAPAAAIAARVAGQTRNITVDPRLFKKRRLRSPRVLFSTQPPREAADTQDLDFEVGGAAPFNRTHRSKRSSSHPIFHRGEFSVCDSVSVWVGDKTTATDIKGKEVMVLGEVNINNSVFKQYFFETKCRDPNPVDSGCRGIDSKHWNSYCTTTHTFVKALTMDGKQAAWWFIRIDTACVCVLSRKAVRRA

SEQ ID NO: 65 - protein, 243 aa, synthetic construct
  REGION 1..243: note = Gp64-19-NGFmut amino acid sequence
MVSAIVLYVLLAAAAHSAFAEPHSESNVPAGHTIPQAHWTKLQHSLDTALRRARSAPAAAIAARVAGQTRNITVDPRLFKKRRLRSPRVLFSTQPPREAADTQDLDFEVGGAAPFNRTHRSKRSSSHPIFHRGEFSVCDSVSVWVGDKTTATDIKGKEVMVLGEVNINNSVFKQYFFETKCRDPNPVDSGCRGIDSKHWNSYCTTTHTFVKALTMDGKQAAWWFIRIDTACVCVLSRKAVRRA

SEQ ID NO: 66 - protein, 241 aa, synthetic construct
  REGION 1..241: note = Alb-19-NGFmut amino acid sequence
MKWVTFISLLFLFSSAYSEPHSESNVPAGHTIPQAHWTKLQHSLDTALRRARSAPAAAIAARVAGQTRNITVDPRLFKKRRLRSPRVLFSTQPPREAADTQDLDFEVGGAAPFNRTHRSKRSSSHPIFHRGEFSVCDSVSVWVGDKTTATDIKGKEVMVLGEVNINNSVFKQYFFETKCRDPNPVDSGCRGIDSKHWNSYCTTTHTFVKALTMDGKQAAWWFIRIDTACVCVLSRKAVRRA

SEQ ID NO: 67 - protein, 50 aa, synthetic construct
  REGION 1..50: note = PDGFR
NAVGQDTQEVIVVPHSLPFKVVVISAILALVVLTIISLIILIMLWQKKPR

SEQ ID NO: 68 - protein, 9 aa, synthetic construct
  REGION 1..9: note = Label Peptide 1st
YPYDVPDYA

SEQ ID NO: 69 - protein, 18 aa, synthetic construct
  REGION 1..18: note = Label Peptide 2nd
YPYDVPDYAYPYDVPDYA

SEQ ID NO: 70 - protein, 253 aa, synthetic construct; identical to SEQ ID NO: 15
  REGION 1..253: note = IGK19-NGFmut amino acid sequence (with label)